European Patent Specification EP 3 757 216 B1, published August 7, 2024. Title: Engineered recombinant Fc gamma RIIa. Applicant: TOSOH Corporation. The sequence listing filed with the application follows.

SEQUENCE LISTING (53 sequences)

SEQ ID NO: 1 - protein, 317 aa, Homo sapiens
  ref <308>: UniProt P12318-1
  ref <309>: 2007-11-13
  ref <313>: (1)..(317)
MTMETQMSQNVCPRNLWLLQPLTVLLLLASADSQAAAPPKAVLKLEPPWINVLQEDSVTLTCQGARSPESDSIQWFHNGNLIPTHTQPSYRFKANNNDSGEYTCQTGQTSLSDPVHLTVLSEWLVLQTPHLEFQEGETIMLRCHSWKDKPLVKVTFFQNGKSQKFSHLDPTFSIPQANHSHSGDYHCTGNIGYTLFSSKPVTITVQVPSMGSSSPMGIIVAVVIATAVAAIVAAVVALIYCRKKRISANSTDPVKAAQFEPPGRQMIAIRKRQLEETNNDYETADGGYMTLNPRAPTDDDKNIYLTLPPNDHVNSNN

SEQ ID NO: 2 - protein, 209 aa, Artificial Sequence
  MalE signal - FcgRIIa - 6His
MKIKTGARILALSALTTMMFSASALAMGQAAAPPKAVLKLEPPWINVLQEDSVTLTCQGARSPESDSIQWFHNGNLIPTHTQPSYRFKANNNDSGEYTCQTGQTSLSDPVHLTVLSEWLVLQTPHLEFQEGETIMLRCHSWKDKPLVKVTFFQNGKSQKFSHLDPTFSIPQANHSHSGDYHCTGNIGYTLFSSKPVTITVQGGHHHHHH

SEQ ID NO: 3 - protein, 209 aa, Artificial Sequence
  MalE signal - FcgRIIa-m6 - 6His
MKIKTGARILALSALTTMMFSASALAMGQAAAPPKAVLKLEPPWINVLQEDSVTLTCQGARSPESDSVQWFHNGNLIPTQTQPTYRFKATSNDSGEYTCQTGQTSLSDPVHLTVLSEWLVLQTPRLEFQEGETIMLRCHSWKDKPLVKVTFFQNGKSQKFSHLDPTFSIPQANHSHSGDYHCTGNIGYTLFSSKPVTITVQGGHHHHHH

SEQ ID NO: 4 - DNA, 627 bp, Artificial Sequence
  DNA encoding MalE signal - FcgRIIa-m6 - 6His
atgaaaataaaaacaggtgcacgcatcctcgcattatccgcattaacgacgatgatgttttccgcctcggctctcgccatgggacaagccgcagcgcctccaaaggcggttctgaaactggagccgccgtggattaatgtgttgcaggaagatagcgtgacgctgacctgccagggagcccgtagcccggaatcagacagcgtacagtggtttcacaacggcaatttgatccccactcaaacgcagccgacgtaccgtttcaaagccaccagtaacgattcgggcgaatatacctgccagacaggccagaccagcctgtcggatccagtgcacctgaccgtgctgtcagaatggctggtgctgcaaaccccgcgtctggaatttcaggaaggcgaaaccataatgctgcgttgccacagctggaaagataaaccgctggtgaaggtcacgttcttccagaacgggaagagccagaagttctcccatctcgacccgacttttagcatcccccaggcgaatcatagccatagcggcgattatcactgcaccgggaatattgggtatacgttgtttagcagcaagccggttactatcaccgtgcagggcggccatcatcatcatcatcat

SEQ ID NO: 5 - protein, 209 aa, Artificial Sequence
  MalE signal - FcgRIIa-m7 - 6His
MKIKTGARILALSALTTMMFSASALAMGQAAAPPKAVLKLEPPWINVLQEDSVTLTCQGARSPESDSVQWFHNGNLIPTQTQPTYRFKATSNDSGEYTCQTGQTSLSDPVHLTVLSEWLVLQTPRLEFQEGETIMLRCHSWKDKPLVKVTFFQNGKSQKFSHLDPTFSIPQANHSHSGDYHCTGNIGYTSFSSKPVTITVQGGHHHHHH

SEQ ID NO: 6 - DNA, 627 bp, Artificial Sequence
  DNA encoding MalE signal - FcgRIIa-m7 - 6His
atgaaaataaaaacaggtgcacgcatcctcgcattatccgcattaacgacgatgatgttttccgcctcggctctcgccatgggacaagccgcagcgcctccaaaggcggttctgaaactggagccgccgtggattaatgtgttgcaggaagatagcgtgacgctgacctgccagggagcccgtagcccggaatcagacagcgtacagtggtttcacaacggcaatttgatccccactcaaacgcagccgacgtaccgtttcaaagccaccagtaacgattcgggcgaatatacctgccagacaggccagaccagcctgtcggatccagtgcacctgaccgtgctgtcagaatggctggtgctgcaaaccccgcgtctggaatttcaggaaggcgaaaccataatgctgcgttgccacagctggaaagataaaccgctggtgaaggtcacgttcttccagaacgggaagagccagaagttctcccatctcgacccgacttttagcatcccccaggcgaatcatagccatagcggcgattatcactgcaccgggaatattgggtatacgtcgtttagcagcaagccggttactatcaccgtgcagggcggccatcatcatcatcatcat

SEQ ID NO: 7 - protein, 209 aa, Artificial Sequence
  MalE signal - FcgRIIa-m1 - 6His
MKIKTGARILALSALTTMMFSASALAMGQAAAPPKAVLKLEPPWINVLQEDSVTLTCQGARSPESDSIQWFHNGNLIPTHTQPSYRFKANNNDSGEYTCQTGQTSLSDPVHLTVLSEWLVLQTPHLEFQEGETIMLRCHSWKDKPLVKVTFFQNGKSQKFSHLDPTFSIPQANHSHSGDYHCTGNIGYTSFSSKPVTITVQGGHHHHHH

SEQ ID NO: 8 - DNA, 20 bp, Artificial Sequence
  Oligonucleotide
taatacgactcactataggg

SEQ ID NO: 9 - DNA, 21 bp, Artificial Sequence
  Oligonucleotide
atgctagttattgctcagcgg

SEQ ID NO: 10 - DNA, 630 bp, Artificial Sequence
  DNA encoding MalE signal - FcgRIIa-m8a (I45T) - 6His
atgaaaataaaaacaggtgcacgcatcctcgcattatccgcattaacgacgatgatgttttccgcctcggctctcgccatgggacaagccgcagcgcctccaaaggcggttctgaaactggagccgccgtggaccaatgtgttgcaggaagatagcgtgacgctgacctgccagggagcccgtagcccggaatcagacagcgtacagtggtttcacaacggcaatttgatccccactcaaacgcagccgacgtaccgtttcaaagccaccagtaacgattcgggcgaatatacctgccagacaggccagaccagcctgtcggatccagtgcacctgaccgtgctgtcagaatggctggtgctgcaaaccccgcgtctggaatttcaggaaggcgaaaccataatgctgcgttgccacagctggaaagataaaccgctggtgaaggtcacgttcttccagaacgggaagagccagaagttctcccatctcgacccgacttttagcatcccccaggcgaatcatagccatagcggcgattatcactgcaccgggaatattgggtatacgtcttttagcagcaagccggttactatcaccgtgcagggcggccatcatcatcatcatcattaa

SEQ ID NO: 11 - protein, 209 aa, Artificial Sequence
  MalE signal - FcRIIa-m8A (I45T) - 6His
MKIKTGARILALSALTTMMFSASALAMGQAAAPPKAVLKLEPPWTNVLQEDSVTLTCQGARSPESDSVQWFHNGNLIPTQTQPTYRFKATSNDSGEYTCQTGQTSLSDPVHLTVLSEWLVLQTPRLEFQEGETIMLRCHSWKDKPLVKVTFFQNGKSQKFSHLDPTFSIPQANHSHSGDYHCTGNIGYTSFSSKPVTITVQGGHHHHHH

SEQ ID NO: 12 - DNA, 630 bp, Artificial Sequence
  DNA encoding MalE signal - FcgRIIa-m8B (Q69L) - 6His
atgaaaataaaaacaggtgcacgcatcctcgcattatccgcattaacgacgatgatgttttccgcctcggctctcgccatgggacaagccgcagcgcctccaaaggcggttctgaaactggagccgccgtggattaatgtgttgcaggaagatagcgtgacgctgacctgccagggagcccgtagcccggaatcagacagcgtactgtggtttcacaacggcaatttgatccccactcaaacgcagccgacgtaccgtttcaaagccaccagtaacgattcgggcgaatatacctgccagacaggccagaccagcctgtcggatccagtgcacctgaccgtgctgtcagaatggctggtgctgcaaaccccgcgtctggaatttcaggaaggcgaaaccataatgctgcgttgccacagctggaaagataaaccgctggtgaaggtcacgttcttccagaacgggaagagccagaagttctcccatctcgacccgacttttagcatcccccaggcgaatcatagccatagcggcgattatcactgcaccgggaatattgggtatacgtcttttagcagcaagccggttactatcaccgtgcagggcggccatcatcatcatcatcattaa

SEQ ID NO: 13 - protein, 209 aa, Artificial Sequence
  MalE signal - FcRIIa-m8B (Q69L) - 6His
MKIKTGARILALSALTTMMFSASALAMGQAAAPPKAVLKLEPPWINVLQEDSVTLTCQGARSPESDSVLWFHNGNLIPTQTQPTYRFKATSNDSGEYTCQTGQTSLSDPVHLTVLSEWLVLQTPRLEFQEGETIMLRCHSWKDKPLVKVTFFQNGKSQKFSHLDPTFSIPQANHSHSGDYHCTGNIGYTSFSSKPVTITVQGGHHHHHH

SEQ ID NO: 14 - DNA, 630 bp, Artificial Sequence
  DNA encoding MalE signal - FcgRIIa-m8C (P83L) - 6His
atgaaaataaaaacaggtgcacgcatcctcgcattatccgcattaacgacgatgatgttttccgcctcggctctcgccatgggacaagccgcagcgcctccaaaggcggttctgaaactggagccgccgtggattaatgtgttgcaggaagatagcgtgacgctgacctgccagggagcccgtagcccggaatcagacagcgtacagtggtttcacaacggcaatttgatccccactcaaacgcagctgacgtaccgtttcaaagccaccagtaacgattcgggcgaatatacctgccagacaggccagaccagcctgtcggatccagtgcacctgaccgtgctgtcagaatggctggtgctgcaaaccccgcgtctggaatttcaggaaggcgaaaccataatgctgcgttgccacagctggaaagataaaccgctggtgaaggtcacgttcttccagaacgggaagagccagaagttctcccatctcgacccgacttttagcatcccccaggcgaatcatagccatagcggcgattatcactgcaccgggaatattgggtatacgtcttttagcagcaagccggttactatcaccgtgcagggcggccatcatcatcatcatcattaa

SEQ ID NO: 15 - protein, 209 aa, Artificial Sequence
  MalE signal - FcgRIIa-m8C (P83L) - 6His
MKIKTGARILALSALTTMMFSASALAMGQAAAPPKAVLKLEPPWINVLQEDSVTLTCQGARSPESDSVQWFHNGNLIPTQTQLTYRFKATSNDSGEYTCQTGQTSLSDPVHLTVLSEWLVLQTPRLEFQEGETIMLRCHSWKDKPLVKVTFFQNGKSQKFSHLDPTFSIPQANHSHSGDYHCTGNIGYTSFSSKPVTITVQGGHHHHHH

SEQ ID NO: 16 - DNA, 630 bp, Artificial Sequence
  DNA encoding MalE signal - FcgRIIa-m8D (T123P) - 6His
atgaaaataaaaacaggtgcacgcatcctcgcattatccgcattaacgacgatgatgttttccgcctcggctctcgccatgggacaagccgcagcgcctccaaaggcggttctgaaactggagccgccgtggattaatgtgttgcaggaagatagcgtgacgctgacctgccagggagcccgtagcccggaatcagacagcgtacagtggtttcacaacggcaatttgatccccactcaaacgcagccgacgtaccgtttcaaagccaccagtaacgattcgggcgaatatacctgccagacaggccagaccagcctgtcggatccagtgcacctgaccgtgctgtcagaatggctggtgctgcaaccgccgcgtctggaatttcaggaaggcgaaaccataatgctgcgttgccacagctggaaagataaaccgctggtgaaggtcacgttcttccagaacgggaagagccagaagttctcccatctcgacccgacttttagcatcccccaggcgaatcatagccatagcggcgattatcactgcaccgggaatattgggtatacgtcttttagcagcaagccggttactatcaccgtgcagggcggccatcatcatcatcatcattaa

SEQ ID NO: 17 - protein, 209 aa, Artificial Sequence
  MalE signal - FcRIIa-m8D (T123P) - 6His
MKIKTGARILALSALTTMMFSASALAMGQAAAPPKAVLKLEPPWINVLQEDSVTLTCQGARSPESDSVQWFHNGNLIPTQTQPTYRFKATSNDSGEYTCQTGQTSLSDPVHLTVLSEWLVLQPPRLEFQEGETIMLRCHSWKDKPLVKVTFFQNGKSQKFSHLDPTFSIPQANHSHSGDYHCTGNIGYTSFSSKPVTITVQGGHHHHHH

SEQ ID NO: 18 - DNA, 630 bp, Artificial Sequence
  DNA encoding MalE signal - FcRIIa-m10A (I45T, Q69L) - 6His
atgaaaataaaaacaggtgcacgcatcctcgcattatccgcattaacgacgatgatgttttccgcctcggctctcgccatgggacaagccgcagcgcctccaaaggcggttctgaaactggagccgccgtggaccaatgtgttgcaggaagatagcgtgacgctgacctgccagggagcccgtagcccggaatcagacagcgtactgtggtttcacaacggcaatttgatccccactcaaacgcagccgacgtaccgtttcaaagccaccagtaacgattcgggcgaatatacctgccagacaggccagaccagcctgtcggatccagtgcacctgaccgtgctgtcagaatggctggtgctgcaaccgccgcgtctggaatttcaggaaggcgaaaccataatgctgcgttgccacagctggaaagataaaccgctggtgaaggtcacgttcttccagaacgggaagagccagaagttctcccatctcgacccgacttttagcatcccccaggcgaatcatagccatagcggcgattatcactgcaccgggaatattgggtatacgtcttttagcagcaagccggttactatcaccgtgcagggcggccatcatcatcatcatcattaa

SEQ ID NO: 19 - protein, 209 aa, Artificial Sequence
  MalE signal - FcRIIa-m10A (I45T, Q69L) - 6His
MKIKTGARILALSALTTMMFSASALAMGQAAAPPKAVLKLEPPWTNVLQEDSVTLTCQGARSPESDSVLWFHNGNLIPTQTQPTYRFKATSNDSGEYTCQTGQTSLSDPVHLTVLSEWLVLQPPRLEFQEGETIMLRCHSWKDKPLVKVTFFQNGKSQKFSHLDPTFSIPQANHSHSGDYHCTGNIGYTSFSSKPVTITVQGGHHHHHH

SEQ ID NO: 20 - DNA, 630 bp, Artificial Sequence
  DNA encoding MalE signal - FcgRIIa-m10B (I45T, P83L) - 6His
atgaaaataaaaacaggtgcacgcatcctcgcattatccgcattaacgacgatgatgttttccgcctcggctctcgccatgggacaagccgcagcgcctccaaaggcggttctgaaactggagccgccgtggaccaatgtgttgcaggaagatagcgtgacgctgacctgccagggagcccgtagcccggaatcagacagcgtacagtggtttcacaacggcaatttgatccccactcaaacgcagctgacgtaccgtttcaaagccaccagtaacgattcgggcgaatatacctgccagacaggccagaccagcctgtcggatccagtgcacctgaccgtgctgtcagaatggctggtgctgcaaccgccgcgtctggaatttcaggaaggcgaaaccataatgctgcgttgccacagctggaaagataaaccgctggtgaaggtcacgttcttccagaacgggaagagccagaagttctcccatctcgacccgacttttagcatcccccaggcgaatcatagccatagcggcgattatcactgcaccgggaatattgggtatacgtcttttagcagcaagccggttactatcaccgtgcagggcggccatcatcatcatcatcattaa

SEQ ID NO: 21 - protein, 209 aa, Artificial Sequence
  MalE signal - FcRIIa-m10B (I45T, P83L) - 6His
MKIKTGARILALSALTTMMFSASALAMGQAAAPPKAVLKLEPPWTNVLQEDSVTLTCQGARSPESDSVQWFHNGNLIPTQTQLTYRFKATSNDSGEYTCQTGQTSLSDPVHLTVLSEWLVLQPPRLEFQEGETIMLRCHSWKDKPLVKVTFFQNGKSQKFSHLDPTFSIPQANHSHSGDYHCTGNIGYTSFSSKPVTITVQGGHHHHHH

SEQ ID NO: 22 - DNA, 630 bp, Artificial Sequence
  DNA encoding MalE signal - FcgRIIa-m10C (Q69L, P83L) - 6His
atgaaaataaaaacaggtgcacgcatcctcgcattatccgcattaacgacgatgatgttttccgcctcggctctcgccatgggacaagccgcagcgcctccaaaggcggttctgaaactggagccgccgtggattaatgtgttgcaggaagatagcgtgacgctgacctgccagggagcccgtagcccggaatcagacagcgtactgtggtttcacaacggcaatttgatccccactcaaacgcagctgacgtaccgtttcaaagccaccagtaacgattcgggcgaatatacctgccagacaggccagaccagcctgtcggatccagtgcacctgaccgtgctgtcagaatggctggtgctgcaaccgccgcgtctggaatttcaggaaggcgaaaccataatgctgcgttgccacagctggaaagataaaccgctggtgaaggtcacgttcttccagaacgggaagagccagaagttctcccatctcgacccgacttttagcatcccccaggcgaatcatagccatagcggcgattatcactgcaccgggaatattgggtatacgtcttttagcagcaagccggttactatcaccgtgcagggcggccatcatcatcatcatcattaa

SEQ ID NO: 23 - protein, 209 aa, Artificial Sequence
  MalE signal - FcgRIIa-m10C (Q69L, P83L) - 6His
MKIKTGARILALSALTTMMFSASALAMGQAAAPPKAVLKLEPPWINVLQEDSVTLTCQGARSPESDSVLWFHNGNLIPTQTQLTYRFKATSNDSGEYTCQTGQTSLSDPVHLTVLSEWLVLQPPRLEFQEGETIMLRCHSWKDKPLVKVTFFQNGKSQKFSHLDPTFSIPQANHSHSGDYHCTGNIGYTSFSSKPVTITVQGGHHHHHH

SEQ ID NO: 24 - DNA, 630 bp, Artificial Sequence
  DNA encoding MalE signal - FcgRIIa-m11 - 6His
atgaaaataaaaacaggtgcacgcatcctcgcattatccgcattaacgacgatgatgttttccgcctcggctctcgccatgggacaagccgcagcgcctccaaaggcggttctgaaactggagccgccgtggaccaatgtgttgcaggaagatagcgtgacgctgacctgccagggagcccgtagcccggaatcagacagcgtactgtggtttcacaacggcaatttgatccccactcaaacgcagctgacgtaccgtttcaaagccaccagtaacgattcgggcgaatatacctgccagacaggccagaccagcctgtcggatccagtgcacctgaccgtgctgtcagaatggctggtgctgcaaccgccgcgtctggaatttcaggaaggcgaaaccataatgctgcgttgccacagctggaaagataaaccgctggtgaaggtcacgttcttccagaacgggaagagccagaagttctcccatctcgacccgacttttagcatcccccaggcgaatcatagccatagcggcgattatcactgcaccgggaatattgggtatacgtcttttagcagcaagccggttactatcaccgtgcagggcggccatcatcatcatcatcattaa

SEQ ID NO: 25 - protein, 209 aa, Artificial Sequence
  MalE signal - FcgRIIa-m11 - 6His
MKIKTGARILALSALTTMMFSASALAMGQAAAPPKAVLKLEPPWTNVLQEDSVTLTCQGARSPESDSVLWFHNGNLIPTQTQLTYRFKATSNDSGEYTCQTGQTSLSDPVHLTVLSEWLVLQPPRLEFQEGETIMLRCHSWKDKPLVKVTFFQNGKSQKFSHLDPTFSIPQANHSHSGDYHCTGNIGYTSFSSKPVTITVQGGHHHHHH

SEQ ID NO: 26 - DNA, 34 bp, Artificial Sequence
  Oligonucleotide I45T - F
ctggagccgccgtggaccaatgtgttgcaggaag

SEQ ID NO: 27 - DNA, 33 bp, Artificial Sequence
  Oligonucleotide I45T - R
ttcctgcaacacattggtccacggcggctccag

SEQ ID NO: 28 - DNA, 33 bp, Artificial Sequence
  Oligonucleotide Q69L - F
gaatcagacagcgtactgtggtttcacaacggc

SEQ ID NO: 29 - DNA, 33 bp, Artificial Sequence
  Oligonucleotide Q69L - R
gccgttgtgaaaccagactacgctgtctgattc

SEQ ID NO: 30 - DNA, 36 bp, Artificial Sequence
  Oligonucleotide P83L - F
actcaaacgcagctgacgtaccgtttcaaagccacc

SEQ ID NO: 31 - DNA, 37 bp, Artificial Sequence
  Oligonucleotide P83L - R
tttgaaacggtacgtcagctgcgtttgagtggggatc

SEQ ID NO: 32 - DNA, 34 bp, Artificial Sequence
  Oligonucleotide T123P - F
tggctggtgctgcaaccgccgcgtctggaatttc

SEQ ID NO: 33 - DNA, 32 bp, Artificial Sequence
  Oligonucleotide T123P - R
aaattccagacgcggcggttgcagcaccagcc

SEQ ID NO: 34 - DNA, 628 bp, Homo sapiens
  DNA encoding MalE signal - FcgRIIa(m11)-Del1 - 6His
atgaaaataaaaacaggtgcacgcatcctcgcattatccgcattaacgacgatgatgttttccgcctcggctctcgccatgggacaagccgcagcgcctccaaaggcggttctgaaactggagccgccgtggaccaatgtgttgcaggaagatagcgtgacgctgacctgccagggagcccgtccggaatcagacagcgtactgtggtttcacaacggcaatttgatccccactcaaacgcagctgacgtaccgtttcaaagccaccagtaacgattcgggcgaatatacctgccagacaggccagaccagcctgtcggatccagtgcacctgaccgtgctgtcagaatggctggtgctgcaaccgccgcgtctggaatttcaggaaggcgaaaccataatgctgcgttgccacagctggaaagataaaccgctggtgaaggtcacgttcttccagaacgggaagagccagaagttctcccatctcgacccgacttttagcatcccccaggcgaatcatagccatagcggcgattatcactgcaccgggaatattgggtatacgtcttttagcagcaagccggttactatcaccgtgcagggcggccatcatcatcatcatcattaag

SEQ ID NO: 35 - protein, 208 aa, Homo sapiens
  MalE signal - FcgRIIa(m11)-Del1 - 6His
MKIKTGARILALSALTTMMFSASALAMGQAAAPPKAVLKLEPPWTNVLQEDSVTLTCQGARPESDSVLWFHNGNLIPTQTQLTYRFKATSNDSGEYTCQTGQTSLSDPVHLTVLSEWLVLQPPRLEFQEGETIMLRCHSWKDKPLVKVTFFQNGKSQKFSHLDPTFSIPQANHSHSGDYHCTGNIGYTSFSSKPVTITVQGGHHHHHH

SEQ ID NO: 36 - DNA, 625 bp, Homo sapiens
  DNA encoding MalE signal - FcgRIIa(m11)-Del2 - 6His
atgaaaataaaaacaggtgcacgcatcctcgcattatccgcattaacgacgatgatgttttccgcctcggctctcgccatgggaactcccgcagcgcctccaaaggcggttctgaaactggagccgcagtggaccaatgtgttgcaggaagatagcgtgacgctgacctgccgtggaacccatccgtcagacagcgtactgtggtttcacaacggcaatttgatccccactcaaacgcagctgacgtaccgtttcaaagccaccagtaacgattcgggcgaatatacctgccagacaggccagaccagcctgtcggatccagtgcacctgaccgtgctgtcagaatggctggtgctgcaaccgccgcgtctggaatttcaggaaggcgaaaccatagtgctgcgttgccacagctggaaagataaaccgctggtgaaggtcacgttcttccagaacgggaagagcaagaagttctcccgtagcgacccgaattttagcatcccccaggcgaatcatagccatagcggcgattatcactgcaccgggaatattgggtatacgtcttatagcagcaagccggttactatcaccgtgcagggcggccatcatcatcatcatcattaag

SEQ ID NO: 37 - protein, 207 aa, Homo sapiens
  MalE signal - FcgRIIa(m11)-Del2 - 6His
MKIKTGARILALSALTTMMFSASALAMGQAAAPPKAVLKLEPPWTNVLQEDSVTLTCQGARPSDSVLWFHNGNLIPTQTQLTYRFKATSNDSGEYTCQTGQTSLSDPVHLTVLSEWLVLQPPRLEFQEGETIMLRCHSWKDKPLVKVTFFQNGKSQKFSHLDPTFSIPQANHSHSGDYHCTGNIGYTSFSSKPVTITVQGGHHHHHH

SEQ ID NO: 38 - DNA, 622 bp, Homo sapiens
  DNA encoding MalE signal - FcgRIIa(m11)-Del3 - 6His
atgaaaataaaaacaggtgcacgcatcctcgcattatccgcattaacgacgatgatgttttccgcctcggctctcgccatgggacaagccgcagcgcctccaaaggcggttctgaaactggagccgccgtggaccaatgtgttgcaggaagatagcgtgacgctgacctgccagggagcccgttcagacagcgtactgtggtttcacaacggcaatttgatccccactcaaacgcagctgacgtaccgtttcaaagccaccagtaacgattcgggcgaatatacctgccagacaggccagaccagcctgtcggatccagtgcacctgaccgtgctgtcagaatggctggtgctgcaaccgccgcgtctggaatttcaggaaggcgaaaccataatgctgcgttgccacagctggaaagataaaccgctggtgaaggtcacgttcttccagaacgggaagagccagaagttctcccatctcgacccgacttttagcatcccccaggcgaatcatagccatagcggcgattatcactgcaccgggaatattgggtatacgtcttttagcagcaagccggttactatcaccgtgcagggcggccatcatcatcatcatcattaag

SEQ ID NO: 39 - protein, 206 aa, Homo sapiens
  MalE signal - FcgRIIa(m11)-Del3 - 6His
MKIKTGARILALSALTTMMFSASALAMGQAAAPPKAVLKLEPPWTNVLQEDSVTLTCQGARSDSVLWFHNGNLIPTQTQLTYRFKATSNDSGEYTCQTGQTSLSDPVHLTVLSEWLVLQPPRLEFQEGETIMLRCHSWKDKPLVKVTFFQNGKSQKFSHLDPTFSIPQANHSHSGDYHCTGNIGYTSFSSKPVTITVQGGHHHHHH

SEQ ID NO: 40 - DNA, 619 bp, Homo sapiens
  DNA encoding MalE signal - FcgRIIa(m11)-Del4 - 6His
atgaaaataaaaacaggtgcacgcatcctcgcattatccgcattaacgacgatgatgttttccgcctcggctctcgccatgggacaagccgcagcgcctccaaaggcggttctgaaactggagccgccgtggaccaatgtgttgcaggaagatagcgtgacgctgacctgccagggagcctcagacagcgtactgtggtttcacaacggcaatttgatccccactcaaacgcagctgacgtaccgtttcaaagccaccagtaacgattcgggcgaatatacctgccagacaggccagaccagcctgtcggatccagtgcacctgaccgtgctgtcagaatggctggtgctgcaaccgccgcgtctggaatttcaggaaggcgaaaccataatgctgcgttgccacagctggaaagataaaccgctggtgaaggtcacgttcttccagaacgggaagagccagaagttctcccatctcgacccgacttttagcatcccccaggcgaatcatagccatagcggcgattatcactgcaccgggaatattgggtatacgtcttttagcagcaagccggttactatcaccgtgcagggcggccatcatcatcatcatcattaag

SEQ ID NO: 41 - protein, 205 aa, Homo sapiens
  MalE signal - FcgRIIa(m11)-Del4 - 6His
MKIKTGARILALSALTTMMFSASALAMGQAAAPPKAVLKLEPPWTNVLQEDSVTLTCQGASDSVLWFHNGNLIPTQTQLTYRFKATSNDSGEYTCQTGQTSLSDPVHLTVLSEWLVLQPPRLEFQEGETIMLRCHSWKDKPLVKVTFFQNGKSQKFSHLDPTFSIPQANHSHSGDYHCTGNIGYTSFSSKPVTITVQGGHHHHHH

SEQ ID NO: 42 - DNA, 616 bp, Homo sapiens
  DNA encoding MalE signal - FcgRIIa(m11)-Del5 - 6His
atgaaaataaaaacaggtgcacgcatcctcgcattatccgcattaacgacgatgatgttttccgcctcggctctcgccatgggacaagccgcagcgcctccaaaggcggttctgaaactggagccgccgtggaccaatgtgttgcaggaagatagcgtgacgctgacctgccagggagccgacagcgtactgtggtttcacaacggcaatttgatccccactcaaacgcagctgacgtaccgtttcaaagccaccagtaacgattcgggcgaatatacctgccagacaggccagaccagcctgtcggatccagtgcacctgaccgtgctgtcagaatggctggtgctgcaaccgccgcgtctggaatttcaggaaggcgaaaccataatgctgcgttgccacagctggaaagataaaccgctggtgaaggtcacgttcttccagaacgggaagagccagaagttctcccatctcgacccgacttttagcatcccccaggcgaatcatagccatagcggcgattatcactgcaccgggaatattgggtatacgtcttttagcagcaagccggttactatcaccgtgcagggcggccatcatcatcatcatcattaag

SEQ ID NO: 43 - protein, 204 aa, Homo sapiens
  MalE signal - FcgRIIa(m11)-Del5 - 6His
MKIKTGARILALSALTTMMFSASALAMGQAAAPPKAVLKLEPPWTNVLQEDSVTLTCQGADSVLWFHNGNLIPTQTQLTYRFKATSNDSGEYTCQTGQTSLSDPVHLTVLSEWLVLQPPRLEFQEGETIMLRCHSWKDKPLVKVTFFQNGKSQKFSHLDPTFSIPQANHSHSGDYHCTGNIGYTSFSSKPVTITVQGGHHHHHH

SEQ ID NO: 44 - DNA, 613 bp, Homo sapiens
  DNA encoding MalE signal - FcgRIIa(m11)-Del6 - 6His
atgaaaataaaaacaggtgcacgcatcctcgcattatccgcattaacgacgatgatgttttccgcctcggctctcgccatgggacaagccgcagcgcctccaaaggcggttctgaaactggagccgccgtggaccaatgtgttgcaggaagatagcgtgacgctgacctgccagggagacagcgtactgtggtttcacaacggcaatttgatccccactcaaacgcagctgacgtaccgtttcaaagccaccagtaacgattcgggcgaatatacctgccagacaggccagaccagcctgtcggatccagtgcacctgaccgtgctgtcagaatggctggtgctgcaaccgccgcgtctggaatttcaggaaggcgaaaccataatgctgcgttgccacagctggaaagataaaccgctggtgaaggtcacgttcttccagaacgggaagagccagaagttctcccatctcgacccgacttttagcatcccccaggcgaatcatagccatagcggcgattatcactgcaccgggaatattgggtatacgtcttttagcagcaagccggttactatcaccgtgcagggcggccatcatcatcatcatcattaag

SEQ ID NO: 45 - protein, 203 aa, Homo sapiens
  MalE signal - FcgRIIa(m11)-Del6 - 6His
MKIKTGARILALSALTTMMFSASALAMGQAAAPPKAVLKLEPPWTNVLQEDSVTLTCQGDSVLWFHNGNLIPTQTQLTYRFKATSNDSGEYTCQTGQTSLSDPVHLTVLSEWLVLQPPRLEFQEGETIMLRCHSWKDKPLVKVTFFQNGKSQKFSHLDPTFSIPQANHSHSGDYHCTGNIGYTSFSSKPVTITVQGGHHHHHH

SEQ ID NO: 46 - DNA, 610 bp, Homo sapiens
  DNA encoding MalE signal - FcgRIIa(m11)-Del7 - 6His
atgaaaataaaaacaggtgcacgcatcctcgcattatccgcattaacgacgatgatgttttccgcctcggctctcgccatgggacaagccgcagcgcctccaaaggcggttctgaaactggagccgccgtggaccaatgtgttgcaggaagatagcgtgacgctgacctgccaggacagcgtactgtggtttcacaacggcaatttgatccccactcaaacgcagctgacgtaccgtttcaaagccaccagtaacgattcgggcgaatatacctgccagacaggccagaccagcctgtcggatccagtgcacctgaccgtgctgtcagaatggctggtgctgcaaccgccgcgtctggaatttcaggaaggcgaaaccataatgctgcgttgccacagctggaaagataaaccgctggtgaaggtcacgttcttccagaacgggaagagccagaagttctcccatctcgacccgacttttagcatcccccaggcgaatcatagccatagcggcgattatcactgcaccgggaatattgggtatacgtcttttagcagcaagccggttactatcaccgtgcagggcggccatcatcatcatcatcattaag

SEQ ID NO: 47 - protein, 202 aa, Homo sapiens
  MalE signal - FcgRIIa(m11)-Del7 - 6His
MKIKTGARILALSALTTMMFSASALAMGQAAAPPKAVLKLEPPWTNVLQEDSVTLTCQDSVLWFHNGNLIPTQTQLTYRFKATSNDSGEYTCQTGQTSLSDPVHLTVLSEWLVLQPPRLEFQEGETIMLRCHSWKDKPLVKVTFFQNGKSQKFSHLDPTFSIPQANHSHSGDYHCTGNIGYTSFSSKPVTITVQGGHHHHHH

SEQ ID NO: 48 - DNA, 607 bp, Homo sapiens
  DNA encoding MalE signal - FcgRIIa(m11)-Del8 - 6His
atgaaaataaaaacaggtgcacgcatcctcgcattatccgcattaacgacgatgatgttttccgcctcggctctcgccatgggacaagccgcagcgcctccaaaggcggttctgaaactggagccgccgtggaccaatgtgttgcaggaagatagcgtgacgctgacctgccagagcgtactgtggtttcacaacggcaatttgatccccactcaaacgcagctgacgtaccgtttcaaagccaccagtaacgattcgggcgaatatacctgccagacaggccagaccagcctgtcggatccagtgcacctgaccgtgctgtcagaatggctggtgctgcaaccgccgcgtctggaatttcaggaaggcgaaaccataatgctgcgttgccacagctggaaagataaaccgctggtgaaggtcacgttcttccagaacgggaagagccagaagttctcccatctcgacccgacttttagcatcccccaggcgaatcatagccatagcggcgattatcactgcaccgggaatattgggtatacgtcttttagcagcaagccggttactatcaccgtgcagggcggccatcatcatcatcatcattaag

SEQ ID NO: 49 - protein, 201 aa, Homo sapiens
  MalE signal - FcgRIIa(m11)-Del8 - 6His
MKIKTGARILALSALTTMMFSASALAMGQAAAPPKAVLKLEPPWTNVLQEDSVTLTCQSVLWFHNGNLIPTQTQLTYRFKATSNDSGEYTCQTGQTSLSDPVHLTVLSEWLVLQPPRLEFQEGETIMLRCHSWKDKPLVKVTFFQNGKSQKFSHLDPTFSIPQANHSHSGDYHCTGNIGYTSFSSKPVTITVQGGHHHHHH

SEQ ID NO: 50 - DNA, 604 bp, Homo sapiens
  DNA encoding MalE signal - FcgRIIa(m11)-Del9 - 6His
atgaaaataaaaacaggtgcacgcatcctcgcattatccgcattaacgacgatgatgttttccgcctcggctctcgccatgggacaagccgcagcgcctccaaaggcggttctgaaactggagccgccgtggaccaatgtgttgcaggaagatagcgtgacgctgacctgccaggtactgtggtttcacaacggcaatttgatccccactcaaacgcagctgacgtaccgtttcaaagccaccagtaacgattcgggcgaatatacctgccagacaggccagaccagcctgtcggatccagtgcacctgaccgtgctgtcagaatggctggtgctgcaaccgccgcgtctggaatttcaggaaggcgaaaccataatgctgcgttgccacagctggaaagataaaccgctggtgaaggtcacgttcttccagaacgggaagagccagaagttctcccatctcgacccgacttttagcatcccccaggcgaatcatagccatagcggcgattatcactgcaccgggaatattgggtatacgtcttttagcagcaagccggttactatcaccgtgcagggcggccatcatcatcatcatcattaag

SEQ ID NO: 51 - protein, 200 aa, Homo sapiens
  MalE signal - FcgRIIa(m11)-Del9 - 6His
MKIKTGARILALSALTTMMFSASALAMGQAAAPPKAVLKLEPPWTNVLQEDSVTLTCQVLWFHNGNLIPTQTQLTYRFKATSNDSGEYTCQTGQTSLSDPVHLTVLSEWLVLQPPRLEFQEGETIMLRCHSWKDKPLVKVTFFQNGKSQKFSHLDPTFSIPQANHSHSGDYHCTGNIGYTSFSSKPVTITVQGGHHHHHH

SEQ ID NO: 52 - DNA, 601 bp, Homo sapiens
  DNA encoding MalE signal - FcgRIIa(m11)-Del10 - 6His
atgaaaataaaaacaggtgcacgcatcctcgcattatccgcattaacgacgatgatgttttccgcctcggctctcgccatgggacaagccgcagcgcctccaaaggcggttctgaaactggagccgccgtggaccaatgtgttgcaggaagatagcgtgacgctgacctgcgtactgtggtttcacaacggcaatttgatccccactcaaacgcagctgacgtaccgtttcaaagccaccagtaacgattcgggcgaatatacctgccagacaggccagaccagcctgtcggatccagtgcacctgaccgtgctgtcagaatggctggtgctgcaaccgccgcgtctggaatttcaggaaggcgaaaccataatgctgcgttgccacagctggaaagataaaccgctggtgaaggtcacgttcttccagaacgggaagagccagaagttctcccatctcgacccgacttttagcatcccccaggcgaatcatagccatagcggcgattatcactgcaccgggaatattgggtatacgtcttttagcagcaagccggttactatcaccgtgcagggcggccatcatcatcatcatcattaag

SEQ ID NO: 53 - protein, 199 aa, Homo sapiens
  MalE signal - FcgRIIa(m11)-Del10 - 6His
MKIKTGARILALSALTTMMFSASALAMGQAAAPPKAVLKLEPPWTNVLQEDSVTLTCVLWFHNGNLIPTQTQLTYRFKATSNDSGEYTCQTGQTSLSDPVHLTVLSEWLVLQPPRLEFQEGETIMLRCHSWKDKPLVKVTFFQNGKSQKFSHLDPTFSIPQANHSHSGDYHCTGNIGYTSFSSKPVTITVQGGHHHHHH